European Patent Specification EP 3 720 428 B1, published January 11, 2023. Title: Ophthalmic topical composition for treating diseases of posterior segment of the eye. Applicant: LABORATORIOS SALVAT, S.A. The sequence listing filed with the application follows.

SEQUENCE LISTING (4 sequences)

SEQ ID NO: 1 - DNA, 20 bp, Artificial
  Forward primer
gtcgtaccactggcattgtg

SEQ ID NO: 2 - DNA, 20 bp, Artificial
  Reverse primer
ctctcagctgtggtggtgaa

SEQ ID NO: 3 - DNA, 20 bp, Artificial
  Forward primer
atctactccaggtcctcttc

SEQ ID NO: 4 - DNA, 18 bp, Artificial
  Reverse primer
gatgcggctgatggtgtg